European Patent Specification EP 3 536 776 B1, published October 25, 2023. Title: Novel vertebrate cells and methods for recombinantly expressing a polypeptide of interest. Applicant: Novartis AG. The sequence listing filed with the application follows.

SEQUENCE LISTING (69 sequences)

SEQ ID NO: 1 - protein, 855 aa, Cricetulus griseus
MGSNRGRKAGGSSKDFGARLKYSSGLENMNGFEEGVEFLPVNNAKKVEKRGPRRCVVLVVLLVSFLFLSLVAGFLVWHFLYSNVRIQKVFNGHLRVTNENFLDAYENSNSTEFKDLANQVKEALKLLYSEVPVLGPYHKRSAVTAFSEGSVIAYYWSEFSIPPHLAEEVDRAMAVERVVTLPPRARALKSFVLTSVVAFPTDPRLLGRTQDNSCNFALHAHGGEVMRFTTPGFPNSPYPAHARCQWVLRGDADSVLSLTFRSFDVAPCDELGNDLVTVYDTLSPMEPHAVVRLCGTYPPSYNLTFLSSQNVFLVTLITNTDRRHPGFEATFFQLPKMRSCGGSLSEAQGLFSSPYYPGHYPPNIDCTWNIKVPNNRNVKVRFKLFYLVDPNIPLGTCPKDYVEINGERYCGEKSQFVVSSNSSKITVRFHSDHSYTDTGFLAEYLSYDSNDPCPGMFMCNTGRCIRKDLRCDGWADCPDYSDEHFCRCNTTHQFMCKNKLCKPLFWVCDNINDCGDGSDEEGCSCPAETFKCSNGKCLPQSQKCDGKDNCGDGSDEASCDRVKVVSCTKYTYRCHNGLCLSKGNPECDGKKDCSDGSDEKNCDCGLRSFTKQARVVGGTNADEGEWPWQVSLHALGQGHLCGASLISPNWLVSAAHCFMDDRNFKYSDHTKWTAFLGLLDQSKRSSTGVQEHKLKRIITHPLFNEITFDYDIALLELEKPAEYSTVVRPICLPDTTHVFPAGKAIWVTGWGHTQEGGTGALILQKGEIRVINQTTCEDLMPQQITPRMMCVGFLSGGVDSCQGDSGGPLSSVETEGRIFQAGVVSWGEGCAQRNKPGVYTRLPAVRDWIKEQTGV

SEQ ID NO: 2 - protein, 855 aa, Homo sapiens [sequence omitted]

SEQ ID NO: 3 - protein, 855 aa, Mus musculus
MGSNRGRKAGGGSQDFGAGLKYNSRLENMNGFEEGVEFLPANNAKKVEKRGPRRWVVLVAVLFSFLLLSLMAGLLVWHFHYRNVRVQKVFNGHLRITNEIFLDAYENSTSTEFISLASQVKEALKLLYNEVPVLGPYHKKSAVTAFSEGSVIAYYWSEFSIPPHLAEEVDRAMAVERVVTLPPRARALKSFVLTSVVAFPIDPRMLQRTQDNSCSFALHAHGAAVTRFTTPGFPNSPYPAHARCQWVLRGDADSVLSLTFRSFDVAPCDEHGSDLVTVYDSLSPMEPHAVVRLCGTFSPSYNLTFLSSQNVFLVTLITNTDRRHPGFEATFFQLPKMSSCGGFLSDTQGTFSSPYYPGHYPPNINCTWNIKVPNNRNVKVRFKLFYLVDPNVPVGSCTKDYVEINGEKYCGERSQFVVSSNSSKITVHFHSDHSYTDTGFLAEYLSYDSNDPCPGMFMCKTGRCIRKELRCDGWADCPDYSDERYCRCNATHQFTCKNQFCKPLFWVCDSVNDCGDGSDEEGCSCPAGSFKCSNGKCLPQSQKCNGKDNCGDGSDEASCDSVNVVSCTKYTYRCQNGLCLSKGNPECDGKTDCSDGSDEKNCDCGLRSFTKQARVVGGTNADEGEWPWQVSLHALGQGHLCGASLISPDWLVSAAHCFQDDKNFKYSDYTMWTAFLGLLDQSKRSASGVQELKLKRIITHPSFNDFTFDYDIALLELEKSVEYSTVVRPICLPDATHVFPAGKAIWVTGWGHTKEGGTGALILQKGEIRVINQTTCEDLMPQQITPRMMCVGFLSGGVDSCQGDSGGPLSSAEKDGRMFQAGVVSWGEGCAQRNKPGVYTRLPVVRDWIKEHTGV

SEQ ID NO: 4 - protein, 855 aa, Rattus norvegicus
MGNNRGRKAGGGSQDFGAGLKYNSRLENMNGFEEGVEFLPVNNAKQVEKRGPRRWVVMVAVVFSFLLLSLMAGLLVWHFHYRNVRIQKVFNGHLRITNENFLDAYENSTSTEFISLASQVKEALKLMYSEVPVLGPYHKKSTVTAFSEGSVIAYYWSEFSIPPHLEEEVDRAMAVERVVTLPPRARALKSFVLTSVVAFPIDPRMLQRTQDNSCSFALHARGRTVTRFTTPGFPNSPYPAHARCQWVLRGDADSVLSLTFRSFDVAPCDGHDSDLVTVYDSLSPMEPHAVVRLCGTFSPSYNLTFLSSQNVFLVTLITNTDRRHPGFEATFFQLPKMSSCGGLLSEAQGTFSSPYYPGHYPPNINCTWNIKVPNNRNVKVRFKLFYLVDPNIPVGSCTKDYVEINGEKFCGERSQFVVSSNSSKITVHFHSDHSYTDTGFLAEYLSYDSNDPCPGMFMCKTGRCIRKDLRCDGWADCPDYSDERHCRCNATHQFMCKNQFCKPLFWVCDSVNDCGDGSDEEGCSCPAGSFKCSNGKCLPQSQQCNGKDDCGDGSDEASCDNVNAVSCTKYTYRCQNGLCLNKGNPECDGKKDCSDGSDEKNCDCGLRSFTKQARVVGGTNADEGEWPWQVSLHALGQGHLCGASLISPDWLVSAAHCFQDETIFKYSDHTMWTAFLGLLDQSKRSASGVQEHKLKRIITHPSFNDFTFDYDIALLELEKPAEYSTVVRPICLPDNTHVFPAGKAIWVTGWGHTKEGGTGALILQKGEIRVINQTTCEELLPQQITPRMMCVGFLSGGVDSCQGDSGGPLSSVEKDGRIFQAGVVSWGEGCAQRNKPGVYTRIPEVRDWIKEQTGV

SEQ ID NO: 5 - protein, 855 aa, Pan troglodytes
  misc_feature (561)..(561): Xaa can be any naturally occurring amino acid
MGSDRARKGGGGPKDFGAGLKYNSRHEKVNGLEEGVEFLPVNNVKKVEKHGPGRWVVLAAVLIGLLLVLLGIGFLVWHLQYRDVRVQKVFNGYMRITNENFVDAYENSNSTEFVSLASKVKDALKLLYSGVPFLGPYHKESAVTAFSEGSVIAYYWSEFSIPQHLVEEAERVMAEERVVMLPPRARSLKSFVVTSVVAFPTDSKTVQRTQDNSCSFGLHARGVELMRFTTPGFPDSPYPAHARCQWALRGDADSVLSLTFRSFDLASCDERGSDLVMVYNTLSPMEPHALVQLCGTYPPSYNLTFHSSQNVLLVTLITNTRRRHPGFEATFFQLPRMRSCGGRLRKAQGTFNSPYYPGHYPPNIDCTWNIEVPNNQHVKVRFKFFYLLEPGVPAGTCPKDYVEINGEKYCGERSQFVVTSNSNKITVRFHSDQSYTDTGFLAEYVSYDSSDPCPGQFTCRTGRCIRKELRCDGWADCTDHSDELNCSCDASHQFTCKNKFCKPLFWVCDSVNDCGDNSDEQGCSCPAQTFRCSNGKCLSKSQQCNGKDDCGDGSDEASCPXVNVVTCTKHTYRCLNGLCLSKGNPECDGKEDCSDGSDEKDCDCGLRSFTRQARVVGGTDADEGEWPWQVSLHALGQGHICGASLISPNWLVSAAHCYIDDRGFRYSDPTQWTAFLGLHDQSQRSAPGVQERRLKRIISHPFFNDFTFDYDIALLELEKPAEYSSMVRPICLPDASHVFPAGKAIWVTGWGHTQYGGTGALILQKGEIRVINQTTCENLLPQQITPRMMCVGFLSGGVDSCQGDSGGPLSSVEADGRIFQAGVVSWGDGCAQRNKPGVYTRLPLFRDWIKENTGV

SEQ ID NO: 6 - DNA, 21 bp, Artificial Sequence
  Matriptase/MT-SP1 - sense sequence of siRNA
gcaagaucacuguucgcuutt

SEQ ID NO: 7 - DNA, 21 bp, Artificial Sequence
  Matriptase/MT-SP1 Antisense sequence of siRNA
aagcgaacagugaucuugctg

SEQ ID NO: 8 - DNA, 21 bp, Artificial Sequence
  C1ra - Sense sequence of siRNA
gaugucuuuucucaaaauatt

SEQ ID NO: 9 - DNA, 21 bp, Artificial Sequence
  C1ra - Antisense sequence of siRNA
uauuuugagaaaagacaucat

SEQ ID NO: 10 - DNA, 21 bp, Artificial Sequence
  Gm5077 - sense sequence of siRNA
cgcugaacgugugauuauutt

SEQ ID NO: 11 - DNA, 21 bp, Artificial Sequence
  Gm5077 - Antisense sequence of siRNA
aauaaucacacguucagcggt

SEQ ID NO: 12 - DNA, 21 bp, Artificial Sequence
  Plat - Sense sequence of siRNA
gaaacaagaugaagacagatt

SEQ ID NO: 13 - DNA, 21 bp, Artificial Sequence
  Plat - Antisense sequence of siRNA
ucugucuucaucuuguuuccc

SEQ ID NO: 14 - DNA, 21 bp, Artificial Sequence
  Prss35 - Sense sequence of siRNA
ggccuuagacuacgacuautt

SEQ ID NO: 15 - DNA, 21 bp, Artificial Sequence
  Prss35 - Antisense sequence of siRNA
auagucguagucuaaggccgg

SEQ ID NO: 16 - DNA, 21 bp, Artificial Sequence
  Matriptase/MT-SP1 - Forward Primer Sequence
cgctgagtacctgtcctacga

SEQ ID NO: 17 - DNA, 23 bp, Artificial Sequence
  Matriptase/MT-SP1 - Reverse Primer Sequence
accgtccagtgttacacatgaac

SEQ ID NO: 18 - DNA, 16 bp, Artificial Sequence
  Matriptase/MT-SP1 Reporter 1 Sequence
ccaatgacccatgccc

SEQ ID NO: 19 - DNA, 20 bp, Artificial Sequence
  C1ra Forward Primer Sequence
acctgcaaacaaggctacca

SEQ ID NO: 20 - DNA, 20 bp, Artificial Sequence
  C1ra Reverse Primer Sequence
tggcaaacagctgtgaagga

SEQ ID NO: 21 - DNA, 15 bp, Artificial Sequence
  C1ra Reporter 1 Sequence
cagcacctggtttcc

SEQ ID NO: 22 - DNA, 24 bp, Artificial Sequence
  Gm5077 Forward Primer Sequence
tgcgaggagccatattactacatg

SEQ ID NO: 23 - DNA, 17 bp, Artificial Sequence
  Gm5077 Reverse Primer Sequence
gcagcgcagcgatactc

SEQ ID NO: 24 - DNA, 16 bp, Artificial Sequence
  Gm5077 Reporter 1 Sequence
ccgccgtgttcttcat

SEQ ID NO: 25 - DNA, 24 bp, Artificial Sequence
  Plat Forward Primer Sequence
agctgacatgggaatactgtgatg

SEQ ID NO: 26 - DNA, 25 bp, Artificial Sequence
  Plat Reverse Primer Sequence
cctttaattcgaaactgtggctgtt

SEQ ID NO: 27 - DNA, 15 bp, Artificial Sequence
  Plat Reporter 1 Sequence
ccgtgctccacctgc

SEQ ID NO: 28 - DNA, 21 bp, Artificial Sequence
  Prss35 Forward Primer Sequence
aggagagcaccacacaaagac

SEQ ID NO: 29 - DNA, 20 bp, Artificial Sequence
  Prss35 Reverse Primer Sequence
acacgagtccactggaagga

SEQ ID NO: 30 - DNA, 16 bp, Artificial Sequence
  Prss35 Reporter 1 Sequence
ccccggacccctcctg

SEQ ID NO: 31 - DNA, 345 bp, Cricetulus griseus
ttttttgcccagtcctggttcttccaaactcacaggtgtcactgaacctccggggctgggaagctattgtcggggagcgtctctgagtcctgaaatatctttctgtttagaacatgaatggctttgaggagggtgtggagtttctgcctgtgaataatgccaagaaagtggagaagcgaggcccccggcgctgtgtggtgcttgtggtcctgctggtcagtttcctctttctctcactcgtggctggcttcctggtgtggcacttcctctgtgagtacagtgggggctgtgggagggcgacagaggggtagtgttctctcttctctcagaggacagaccaaaggg

SEQ ID NO: 32 - DNA, 20 bp, Artificial Sequence
  Forward Primer Sequence
ttttttgcccagtcctggtt

SEQ ID NO: 33 - DNA, 20 bp, Artificial Sequence
  Reverse Primer Sequence
ccctttggtctgtcctctga

SEQ ID NO: 34 - DNA, 20 bp, Artificial Sequence
  Cut. Primer
gtggagtttctgcctgtgaa

SEQ ID NO: 35 - DNA, 160 bp, Cricetulus griseus
aacatgaatggctttgaggagggtgtggagtttctgcctgtgaataatgccaagaaagtggagaagcgaggcccccggcgctgtgtggtgcttgtggtcctgctggtcagtttcctctttctctcactcgtggctggcttcctggtgtggcacttcctct

SEQ ID NO: 36 - DNA, 156 bp, Cricetulus griseus
aacatgaatggctttgaggagggtgtggagttcctgtgaataatgccaagaaagtggagaagcgaggcccccggcgctgtgtggtgcttgtggtcctgctggtcagtttcctctttctctcactcgtggctggcttcctggtgtggcacttcctct

SEQ ID NO: 37 - DNA, 156 bp, Cricetulus griseus
aacatgaatggctttgaggagggtgtggagtttctgtgaataatgccaagaaagtggagaagcgaggcccccggcgctgtgtggtgcttgtggtcctgctggtcagtttcctctttctctcactcgtggctggcttcctggtgtggcacttcctct

SEQ ID NO: 38 - DNA, 143 bp, Cricetulus griseus
aacatgaatggctttgaggagggtgaataatgccaagaaagtggagaagcgaggcccccggcgctgtgtggtgcttgtggtcctgctggtcagtttcctctttctctcactcgtggctggcttcctggtgtggcacttcctct

SEQ ID NO: 39 - DNA, 17 bp, Cricetulus griseus
tggagtttctgcctgtg

SEQ ID NO: 40 - DNA, 146 bp, Cricetulus griseus
aacatgaatggctttgaggagggtgtggaataatgccaagaaagtggagaagcgaggcccccggcgctgtgtggtgcttgtggtcctgctggtcagtttcctctttctctcactcgtggctggcttcctggtgtggcacttcctct

SEQ ID NO: 41 - DNA, 14 bp, Cricetulus griseus
gtttctgcctgtga

SEQ ID NO: 42 - DNA, 156 bp, Cricetulus griseus
aacatgaatggctttgaggagggtgtggagtgcctgtgaataatgccaagaaagtggagaagcgaggcccccggcgctgtgtggtgcttgtggtcctgctggtcagtttcctctttctctcactcgtggctggcttcctggtgtggcacttcctct

SEQ ID NO: 43 - DNA, 149 bp, Cricetulus griseus
aacatgaatggctttgaggagggtgtggagtaataatgccaagaaagtggagaagcgaggcccccggcgctgtgtggtgcttgtggtcctgctggtcagtttcctctttctctcactcgtggctggcttcctggtgtggcacttcctct

SEQ ID NO: 44 - DNA, 11 bp, Cricetulus griseus
ttctgcctgtg

SEQ ID NO: 45 - DNA, 153 bp, Cricetulus griseus
aacatgaatggctttgaggagggtgtgggcctgtgaataatgccaagaaagtggagaagcgaggcccccggcgctgtgtggtgcttgtggtcctgctggtcagtttcctctttctctcactcgtggctggcttcctggtgtggcacttcctct

SEQ ID NO: 46 - DNA, 145 bp, Cricetulus griseus
aacatgaatggctttgaggagggtgtgaataatgccaagaaagtggagaagcgaggcccccggcgctgtgtggtgcttgtggtcctgctggtcagtttcctctttctctcactcgtggctggcttcctggtgtggcacttcctct

SEQ ID NO: 47 - DNA, 15 bp, Cricetulus griseus
gagtttctgcctgtg

SEQ ID NO: 48 - protein, 124 aa, Cricetulus griseus
MGSNRGRKAGGSSKDFGARLKYSSGLENMNGFEEGVEFLPVNNAKKVEKRGPRRCVVLVVLLVSFLFLSLVAGFLVWHFLYSNVRIQKVFNGHLRVTNENFLDAYENSNSTEFKDLANQVKEAL

SEQ ID NO: 49 - protein, 39 aa, Cricetulus griseus
MGSNRGRKAGGSSKDFGARLKYSSGLENMNGFEEGVEFL

SEQ ID NO: 50 - protein, 52 aa, Cricetulus griseus
IMPRKWRSEAPGAVWCLWSCWSVSSFSHSWLASWCGTSSTQMFGSKRSSMVI

SEQ ID NO: 51 - protein, 25 aa, Cricetulus griseus
GSQMRTFWMPMRTQTPQSSKTWPTR

SEQ ID NO: 52 - protein, 39 aa, Cricetulus griseus; identical to SEQ ID NO: 49

SEQ ID NO: 53 - protein, 52 aa, Cricetulus griseus; identical to SEQ ID NO: 50

SEQ ID NO: 54 - protein, 25 aa, Cricetulus griseus
GSQMRTFWMPMRTQTPQSSKTWPTR

SEQ ID NO: 55 - protein, 36 aa, Cricetulus griseus
MGSNRGRKAGGSSKDFGARLKYSSGLENMNGFEEGE

SEQ ID NO: 56 - protein, 55 aa, Cricetulus griseus
CQESGEARPPALCGACGPAGQFPLSLTRGWLPGVALPLLKCSDPKGLQWSSEGHK

SEQ ID NO: 57 - protein, 6 aa, Cricetulus griseus
ELSGCL

SEQ ID NO: 58 - protein, 23 aa, Cricetulus griseus
ELKLHRVQRPGQPGEGSAEAVVQ

SEQ ID NO: 59 - protein, 37 aa, Cricetulus griseus
MGSNRGRKAGGSSKDFGARLKYSSGLENMNGFEEGVE

SEQ ID NO: 60 - protein, 55 aa, Cricetulus griseus; identical to SEQ ID NO: 56

SEQ ID NO: 61 - protein, 6 aa, Cricetulus griseus
ELSGCL

SEQ ID NO: 62 - protein, 23 aa, Cricetulus griseus
ELKLHRVQRPGQPGEGSAEAVVQ

SEQ ID NO: 63 - protein, 39 aa, Cricetulus griseus
MGSNRGRKAGGSSKDFGARLKYSSGLENMNGFEEGVECL

SEQ ID NO: 64 - protein, 52 aa, Cricetulus griseus; identical to SEQ ID NO: 50

SEQ ID NO: 65 - protein, 25 aa, Cricetulus griseus
GSQMRTFWMPMRTQTPQSSKTWPTR

SEQ ID NO: 66 - protein, 37 aa, Cricetulus griseus; identical to SEQ ID NO: 59

SEQ ID NO: 67 - protein, 55 aa, Cricetulus griseus; identical to SEQ ID NO: 56

SEQ ID NO: 68 - protein, 6 aa, Cricetulus griseus
ELSGCL

SEQ ID NO: 69 - protein, 23 aa, Cricetulus griseus
ELKLHRVQRPGQPGEGSAEAVVQ